European Patent Specification EP 3 625 349 B1, published August 28, 2024. Title: MODIFIED VIRUSES. Applicant: Mayo Foundation for Medical Education and Research. The sequence listing filed with the application follows.

SEQUENCE LISTING (15 sequences)

SEQ ID NO: 1 - protein, 617 aa, measles virus
MSPQRDRINAFYKDNPHPKGSRIVINREHLMIDRPYVLLAVLFVMFLSLIGLLAIAGIRLHRAAIYTAEIHKSLSTNLDVTNSIEHQVKDVLTPLFKIIGDEVGLRTPQRFTDLVKLISDKIKFLNPDREYDFRDLTWCINPPERIKLDYDQYCADVAAEELMNALVNSTLLETRTTNQFLAVSKGNCSGPTTIRGQFSNMSLSLLDLYLGRGYNVSSIVTMTSQGMYGGTYLVEKPNLSSKRSELSQLSMYRVFEVGVIRNPGLGAPVFHMTNYLEQPVSNDLSNCMVALGELKLAALCHGEDSITIPYQGSGKGVSFQLVKLGVWKSPTDMQSWVPLSTDDPVIDRLYLSSHRGVIADNQAKWAVPTTRTDDKLRMETCFQQACKGKIQALCENPEWAPLKDNRIPSYGVLSVDLSLTVELKIKIASGFGPLITHGSGMDLYKSNHNNVYWLTIPPMKNLALGVINTLEWIPRFKVSPYLFTVPIKEAGEDCHAPTYLPAEVDGDVKLSSNLVILPGQDLQYVLATYDTSRVEHAVVYYVYSPSRSFSYFYPFRLPIKGVPIELQVECFTWDQKLWCRHFCVLADSESGGHITHSGMVGMGVSCTVTREDGTNRR

SEQ ID NO: 2 - DNA, 1854 bp, measles virus
atgtcaccgcaaagagaccggataaatgccttctacaaagataacccttatcccaagggaagtaggatagttattaacagagaacatcttatgattgacagaccctatattctgctggctgttctgttcgtcatgtttctgagcttgatcggattgctggcaattgcaggcattagacttcatcgggcagccatctacaccgcggagatccataaaagcctcagtaccaatctagatgtgactaactcaatcgagcatcaggtcaaggacgtgctgacaccactctttaaaatcatcggggatgaagtgggcctgagaacacctcagagattcactgacctagtgaaattcatctctgacaagattaaattccttaatccggatagggagtacgacttcagagatctcacttggtgcatcaacccgccagagaggatcaaactagattatgatcaatactgtgcagatgtggctgctgaagagctcatgaatgcattggtgaactcaactctactggagaccagaacaaccaatcagttcctagctgtctcaaagggaaactgctcagggcccactacaatcagaggtcaattctcaaacatgtcgctgtccttgttggacttgtacttaggtcgaggttacaatgtgtcatctatagtcactatgacatcccagggaatgtatgggggaacctacctagtggaaaagcctaatctgaacagcaaagggtcagagttgtcacaactgagcatgtaccgagtgtttgaagtaggtgttatcagaaacccgggtttgggggctccggtgttccatatgacaaactattttgagcaaccagtcagtaatggtctcggcaactgtatggtggctttgggggagctcaaactcgcagccctttgtcacggggacgattctatcacaattccctatcagggatcagggaaaggtgtcagcttccagctcgtcaagctgggtgtctggaaatccccaaccgacatgcaatcctgggtccccttatcaacggatgatccagtggtagacaggctttacctctcatctcacagaggtgtcatcgctgacaatcaagcaaaatgggctgtcccgacaacacgaacagatgacaagttgcgaatggagacatgcttccagcaggcgtgtaaaggtaaaatccaagcactctgcgagaatcccgagtgggtgccattgaaggataacaggattccttcatacggggtcctgtctgttgatctgagtctgacagttgagcttaaaatcaaaattgcttcgggattcgggccattgatcacacacggctcagggatggacctatacaaatccaaccgcaacaatgtgtattggctgactattccgccaatgagaaatctagccttaggcgtaatcaacacattggagtggataccgagattcaaggttagtcccaacctcttcactgtcccaattaaggaagcaggcgaggactgccatgccccaacatacctacctgcggaggtggacggtgatgtcaaactcagttccaacctggtgattctacctggtcaagatctccaatatgttttggcaacctacgatacctccagggttgagcatgctgtggtttattacgtttacagcccaagccgctcattttcttacttttatccttttaggttgcctataaagggggtcccaatcgaactacaagtggaatgcttcacatgggaccaaaaactctggtgccgtcacttctgtgtgcttgcggactcagaatccggcggacatatcactcactctgggatggtgggcatgggagtcagctgcacagctacccgggaagatggaaccaatcgcagataa

SEQ ID NO: 3 - protein, 617 aa, Artificial Sequence
  construct sequence
MSPQRDRINAFYKDNPHSKGSRIVINREHLMIDRPYVLLAVLFVMFLSLIGLLAIAGIRLHRAAIYTAEIHKSLSTNLDVTNSIEHQVKDVLTPLFKIIGDEVGLRTPQRFTDLVKFISDKIKFLNPDREYDFRDLTWCINPPERIKLNYDQYCADVAAEELMNALVNSTLLETRTTNQFLAVSKGNCPGPTTIRGQFSNMSLSLLDLYLSRGYNVSSIVTMTSQGMYGGTYLVGKPDLNSKGSELSQPSMYRVFEVGVIRNPGLGAPVFHMTNYFEQPISKDLSNCMVALGELKLAALCHRGDSITIPCRGSGKGVSFQLVKLGVWKSPTDMHSWVPLSTDDPVIDRLYLSSHRGVITDNQANWAVPTTRTDDKLQKETCFQQACKGKIQALCENLEWAPLKDSRIPSYGVLSVNLSLAAEPKIKIASGFGPLITHGSGMDLYKSNHNNVYWLTIPPMKNLALGVINTLEWIPRLKVSPYLFTVPIEEADEDCRAPTYLPAEVTGDVKLSSNLVILPGQDLQYVLATYDTSGVEHAVVYYVYSPGGSFSYVYPFRLPIKGTPIELQVECFTWAQRLWCRHFCVLADSESGGHLTHSGMVGMEVSCTVNREDEANRR

SEQ ID NO: 4 - protein, 553 aa, measles virus
MSIMGLKVNVSAIFMAVLLTLQTPTGQIHWGNLSKIGVVGIGSASYKVMTRSSHQSLVIKLMPNITLLNNCTRVEIAEYRRLLRTVLEPIRDALNAMTQNIRPVQSVASSRRHKRFAGVVLAGAALGVATAAQITAGIALHQSMLNSQAIDNLRASLETTNQAIETIRQAGQEMILAVQGVQDYINNELIPSMNQLSCDLIGQKLGLKLLRYYTEILSLFGPSLRDPISAEISIQALSYALGGDINKVLEKLGYSGGDLLGILESGGIKARITHVDTESYFIVLSIAYPTLSEIKGVIVHRLEGVSYNIGSQEWYTTVPKYVATQGYLISNFDESSCTFMPEGTVCSQNALYPMSPLLQECLRGYTKSCARTLVSGSFGNRFILSQGNLIANCASILCKCYTTGTIINQDPDKILTYIAADHCPVVEVNGVTIQVGSRRYPDAVYLHRIDLGPPISLERLDVGTNLGNAIAKLEDAKELLESSDQILRSMKGLSSTSIVYILIAVCLGGLIGIPALICCCRGRCNKKGEQVGMSRPGLKPDLTGTSKSYVRSL

SEQ ID NO: 5 - protein, 1653 aa, measles virus
ATGGGTCTCAAGGTGAACGTCTCTGCCGTATTCATGGCAGTACTGTTAACTCTCCAAACACCCGCCGGTCAAATTCATTGGGGCAATCTCTCTAAGATAGGGGTAGTAGGAATAGGAAGTGCAAGCTACAAAGTTATGACTCGTTCCAGCCATCAATCATTAGTCATAAAATTAATGCCCAATATAACTCTCCTCAATAACTGCACGAGGGTAGAGATTGCAGAATACAGGAGACTACTAAGAACAGTTTTGGAACCAATTAGGGATGCACTTAATGCAATGACCCAGAACATAAGGCCGGTTCAGAGCGTAGCTTCAAGTAGGAGACACAAGAGATTTGCGGGAGTAGTCCTGGCAGGTGCGGCCCTAGGTGTTGCCACAGCTGCTCAGATAACAGCCGGCATTGCACTTCACCGGTCCATGCTGAACTCTCAGGCCATCGACAATCTGAGAGCGAGCCTGGAAACTACTAATCAGGCAATTGAGGCAATCAGACAAGCAGGGCAGGAGATGATATTGGCTGTTCAGGGTGTCCAAGACTACATCAATAATGAGCTGATACCGTCTATGAACCAGCTATCTTGTGATCTAATCGGTCAGAAGCTCGGGCTCAAATTGCTTAGATACTATACAGAAATCCTGTCATTATTTGGCCCCAGCCTACGGGACCCCATATCTGCGGAGATATCTATCCAGGCTTTGAGTTATGCACTTGGAGGAGATATCAATAAGGTGTTAGAAAAGCTCGGATACAGTGGAGGCGATTTACTAGGCATCTTAGAGAGCAGAGGAATAAAGGCTCGGATAACTCACGTCGACACAGAGTCCTACTTCATAGTCCTCAGTATAGCCTATCCGACGCTGTCCGAGATTAAGGGGGTGATTGTCCACCGGCTAGAGGGGGTCTCGTACAACATAGGCTCTCAAGAGTGGTATACCACTGTGCCCAAGTATGTTGCAACCCAAGGGTACCTTATCTCGAATTTTGATGAGTCATCATGTACTTTCATGCCAGAGGGGACTGTGTGCAGCCAAAATGCCTTGTACCCGATGAGTCCTCTGCTCCAAGAATGCCTCCGGGGGTCCACCAAGTCCTGTGCTCGTACACTCGTATCCGGGTCTTTTGGGAACCGGTTCATTTTATCACAAGGGAACCTAATAGCCAATTGTGCATCAATTCTTTGTAAGTGTTACACAACAGGTACGATTATTAATCAAGACCCTGACAAGATCCTAACATACATTGCTGCCGATCGCTGCCCGGTAGTCGAGGTGAACGGCGTGACCATCCAAGTCGGGAGCAGGAGGTATCCAGACGCTGTGTACTTGCACAGAATTGACCTCGGTCCTCCCATATCATTGGAGAGGTTGGACGTAGGGACAAATCTGGGGAATGCAATTGCCAAATTGGAGGATGCCAAGGAATTGTTGGAATCATCGGACCAGATATTGAGAAGTATGAAAGGTTTATCGAGCACTAGCATAGTCTACATCCTGATTGCAGTGTGTCTTGGAGGGTTGATAGGGATCCCCACTTTAATATGTTGCTGCAGGGGGCGTTGTAACAAAAAGGGAGAACAAGTTGGTATGTCAAGACCAGGCCTAAAGCCTGACCTTACAGGAACATCAAAATCCTATGTAAGATCGCTTTGA

SEQ ID NO: 6 - protein, 662 aa, canine distemper virus
MHNKNPKKSKPLPHTRQDPLQQHSTRSAETKTSQGQHSTTSAQRSTYHGPRTSDRSVHYIMNRTRSCKQTSHRSDNIPPHRDHEGIIHHTPESVTQGASSWFKRRQSNATNAGSQYTWLVLWCIGIASLLLCSKAQIHWNNLSTIGIIGTDSVHYKIMTRPSHQYLVIKLMPNVSLIDNCTKAELGEYEKLLNSVLEPINQALTLMTNNVKPLQSVGSGRRQRRFAGVVLAGAALGVATAAQITAGIALHQSNLNAQAIQSLRTSLEQSNKAIEEIREATQETVIAVQGVQDYVNNELVPAMQHMSCELVGQRLGLKLLRYYTELLSIFGPSLRDPISAEISIQALSYALGGEIHKILEKLGYSGNDMIAILESRGIKTKITHVDLPGKLIILSISYPTLSEVKGVIVHRLEAVSYNIGSQEWYTTVPKYVATNGYLISNFDESSCVFVSESAICSQNSLYPMSPILQQCIRGDTSSCARTLVSGTMGNKFILSKGNIVANCASILCKCYSTSTIINQSPDKLLTFIASDTCPLVEIDGVTIQVGGRQYPDMVYESKVALGPAISLERLDVGTNLGNALKKLDDAKVLIDSSNQILETVKRSSFNFGSLLSVPILICTALALLLLIYCCKRRYRQTFKHNTKVDPTFKPDLTGTSKSYVRSL

SEQ ID NO: 7 - protein, 662 aa, canine distemper virus
MHNKIPKRSKPLPHTRQDPLQQHSTRFGETTTSQGRHSTTSAQRSTHHGPRTSDRPVHHTMNRTRSCKQTSHRSDNILPHRDHKGIIHHTPESVTQGASSWFKRRQFNATNAGSQCTWLVLWCIGIASLFLCSKAQIHWNNLSTIGIIGTDSVHYKIMTRPSHQYLVIKLMPNVSLIDNCTKAELGEYEKLLNSVLEPINQALTLMTNNVKPLQSVGSGRRQRRFAGVVLAGAALGVATAAQITAGIALHQSNLNAQAIQSLRTSLEQSNKAIEEIREATQETVIAVQGVQDYVNNELVPAMQHMSCELVGQRLGLKLLRYYTELLSIFGPSLRDPISAEISIQALSYALGGEIHKILEKLGYSGNDMIAILESRGIKTKITHVDLPGKLIILSISYPTLSEVKGVIVHRLETVSYNIGSQEWYTTVPKYVATNGYLISNFDESSCVFFSESAICSQNSLYPMSPILQQCIRGDTSSCARTLVSGTMGNKFILSKGNIVANCASILCKCYSTSTIINQSPDKLLTFIASDTCPLVEIDGVTIQVGGRQYPDMVYESKVALGPAISLERLDVGTNLGNALKKLDDAKVLIDSSNQILETVKRSSFNFGSLLSIPILICTALVLLLLIYCCNRRYRQTFKHNTKVDPTFKPDLTGTSKSYVRSL

SEQ ID NO: 8 - protein, 604 aa, canine distemper virus
MLPYQDKVGAFYKDNARANSTKLSLVTEGHGGRRPPYLLFVLLILLVGILALLAITGVRFHQVSTSNMEFSRLLKEDMEKSEAVHHQVIDVLTPLFKIIGDEIGLRLPQKLNEIKQFILQKTNFFNPNREFDFRDLHWCINPPSTVKVNFTNYCESIGIRKAIASAANPILLSALSGGRGDIFPPHRCSGATTSVGKVFPLSVSLSMSLISRTSEVINMLTAISDGVYGKTYLLVPDDIEREFDTREIRVFEIGFIKRWLNDMPLLQTTNYMVLPKNSKAKVCTIAVGELTLASLCVEESTVLLYHDSSGSQDGILVVTLGIFWATPMDHIEEVIPVAHPSMKKIHITNHRGFIKDSIATWMVPALASEKQEEQKGCLESACQRKTYPMCNQASWEPFGGRQLPSYGRLTLPLDASVDLQLNISFTYGPVILNGDGMDYYESPLLNSGWLTIPPKDGTISGLINKAGRGDQFTVLPHVLTFAPRESSGNCYLPIQTSQIRDRDVLIESNIVVLPTQSIRYVIATYDISRSDHAIVYYVYDPIRTISYTHPFRLTTKGRPDFLRIECFVWDDNLWCHQFYRFEADIANSTTSVENLVRIRFSCNR

SEQ ID NO: 9 - protein, 617 aa, measles virus
MSPQRDRINAFYKDNPHSKGSRIVINREHLMIDRPYVLLAVLFVMFLSLIGLLAIAGIRLHRAAIYTAEIHKSLSTNLDVTNSIEHQVKDVLTPLFKIIGDEVGLRTPQRFTDLVKFISDKIKFLNPDREYDFRDLTWCINPPERIKLNYDQYCADVAAEELMNALVNSTLLETRTTNQFLAVSKGNCSGPTTIRGQFSNMSLSLLDLYLSRGYNVSSIVTMTSQGMYGGTYLVEKPNLNSKGSELSQLSMYRVFEVGVIRNPGLGAPVFHMTNYFEQPISKDLSNCMVALGELKLAALCHGGDSITIPYQGSGKGVSFQLVKLGVWKSPTDMHSWVPLSTDDPVIDRLYLSSHRGVITDNQANWAVPTTRTDDKLRMETCFQQACKGKIQALCENLEWAPLKDSRIPSYGVLSVDLSLAAEPKIKIASGFGPLITHGSGMDLYKSNHNNVYWLTIPPMKNLALGVINTLEWIPRLKVSPNLFTVPIKEAGEDCHAPTYLPAEVDGDVKLSSNLVILPGQDLQYVLATYDTSRVEHAVVYYVYSPSRSFSYFYPFRLPIKGTPIELQVECFTWAQRLWCRHFCVLADSESGGHLTHSGMVGMEVSCTVNREDEANRR

SEQ ID NO: 10 - DNA, 6 bp, Artificial Sequence
  construct sequence
gggaga

SEQ ID NO: 11 - DNA, 17 bp, Artificial Sequence
  construct sequence
taatacgactcactata

SEQ ID NO: 12 - DNA, 68 bp, Artificial Sequence
  construct sequence
taatacgactcactatagggagatgtttggtctgatgaggccgaaaggccgaaactccgtaaggagtc

SEQ ID NO: 13 - DNA, 70 bp, Artificial Sequence
  construct sequence
taatacgactcactatagggagatttggtctgatgagtccgtgaggacgaaacggagtctagactccgtc

SEQ ID NO: 14 - DNA, 70 bp, Artificial Sequence; identical to SEQ ID NO: 13
  construct sequence

SEQ ID NO: 15 - protein, 21 aa, Artificial Sequence
  construct sequence
KNLALGVINTLEWIPRFKVSP